European Patent Specification EP 3 728 286 B1, published July 3, 2024. Title: ENGINEERED O-GLYCOSYLATION IN RECOMBINANT POLYPEPTIDES AND USES THEREOF. Applicant: MedImmune Limited. The sequence listing filed with the application follows.

SEQUENCE LISTING (43 sequences)

SEQ ID NO: 1 - protein, 27 aa, Artificial Sequence
  i0
EFIAWLVKGAAAGGSGSTASSGSGSAT

SEQ ID NO: 2 - protein, 19 aa, Artificial Sequence
  i1
KNPLPTKETIEQEKQAGES

SEQ ID NO: 3 - protein, 19 aa, Artificial Sequence
  i1+10T
KNPLPTKETIEQEKQTGES

SEQ ID NO: 4 - protein, 14 aa, Artificial Sequence
  i2
KNPLPTKETIEQEK

SEQ ID NO: 5 - protein, 20 aa, Artificial Sequence
  i1-11T
  MISC_FEATURE (2)..(6): X is any amino acid
TXXXXXKNPLPTKEAIEQEK

SEQ ID NO: 6 - protein, 11 aa, Artificial Sequence
  i3
KNPLPTKETIE

SEQ ID NO: 7 - protein, 9 aa, Artificial Sequence
  i4
KNPLPTKET

SEQ ID NO: 8 - protein, 6 aa, Artificial Sequence
  i6
PLPTKE

SEQ ID NO: 9 - protein, 6 aa, Artificial Sequence
  i6 +1A
PLPTAE

SEQ ID NO: 10 - protein, 7 aa, Artificial Sequence
  i6 +3P
PLPTKEP

SEQ ID NO: 11 - protein, 7 aa, Artificial Sequence
  i6 dbl
PLPTAEP

SEQ ID NO: 12 - protein, 5 aa, Artificial Sequence
  i7 dbl
PTAEP

SEQ ID NO: 13 - protein, 5 aa, Artificial Sequence
  i8 P-1A
ATAEP

SEQ ID NO: 14 - protein, 5 aa, Artificial Sequence
  O-linked glycosylation sequence
PTAEA

SEQ ID NO: 15 - protein, 9 aa, Artificial Sequence
  O-linked glycosylation sequence
AAPGPTPGP

SEQ ID NO: 16 - protein, 9 aa, Artificial Sequence
  O-linked glycosylation sequence
AAVGATVEG

SEQ ID NO: 17 - protein, 9 aa, Artificial Sequence
  O-linked glycosylation sequence
AADSTTPAP

SEQ ID NO: 18 - protein, 9 aa, Artificial Sequence
  O-linked glycosylation sequence
AASLPSISS

SEQ ID NO: 19 - protein, 20 aa, Artificial Sequence
  O-glycosylation of GLP-1:Fc fusion protein
KGAAAGGSGSTASSGSGSAT

SEQ ID NO: 20 - protein, 33 aa, Artificial Sequence
  O-glycosylation of GLP-1:Fc fusion protein
KGKNPLPTKETIEQEKQAGESAAAGSSGSGSAT

SEQ ID NO: 21 - protein, 33 aa, Artificial Sequence
  O-glycosylation of GLP-1:Fc fusion protein
KGKNPLPTKETIEQEKQTGESAAAGSSGSGSAT

SEQ ID NO: 22 - protein, 28 aa, Artificial Sequence
  O-glycosylation of GLP-1:Fc fusion protein
KGKNPLPTKETIEQEKGSTASSGSGSAT

SEQ ID NO: 23 - protein, 28 aa, Artificial Sequence
  O-glycosylation of GLP-1:Fc fusion protein
KGKNPLPTKETIEQEKGSTASSGSGSAT

SEQ ID NO: 24 - protein, 28 aa, Artificial Sequence
  O-glycosylation of GLP-1:Fc fusion protein
KGKNPLPTKEAIEQEKGSTASSGSGSAT

SEQ ID NO: 25 - protein, 28 aa, Artificial Sequence
  O-glycosylation of GLP-1:Fc fusion protein
KGKNPLPTKETIEQEKGAAASSGSGSAT

SEQ ID NO: 26 - protein, 25 aa, Artificial Sequence
  O-glycosylation of GLP-1:Fc fusion protein
KGKNPLPTKETIEGSTASSGSGSAT

SEQ ID NO: 27 - protein, 25 aa, Artificial Sequence
  O-glycosylation of GLP-1:Fc fusion protein
KGKNPLPTKETGSTASSGSGSGSAT

SEQ ID NO: 28 - protein, 22 aa, Artificial Sequence
  O-glycosylation of GLP-1:Fc fusion protein
KGKNPLPTKEGSTASSGSGSAT

SEQ ID NO: 29 - protein, 12 aa, Artificial Sequence
  O-glycosylation of GLP-1:Fc fusion protein
KGPLPTKEGSAT

SEQ ID NO: 30 - protein, 12 aa, Artificial Sequence
  O-glycosylation of GLP-1:Fc fusion protein
KGPLPTAEGSAT

SEQ ID NO: 31 - protein, 13 aa, Artificial Sequence
  O-glycosylation of GLP-1:Fc fusion protein
KGPLPTKEPGSAT

SEQ ID NO: 32 - protein, 13 aa, Artificial Sequence
  O-glycosylation of GLP-1:Fc fusion protein
KGPLPTAEPGSAT

SEQ ID NO: 33 - protein, 11 aa, Artificial Sequence
  O-glycosylation of GLP-1:Fc fusion protein
KGPTKERGSAT

SEQ ID NO: 34 - protein, 11 aa, Artificial Sequence
  O-glycosylation of GLP-1:Fc fusion protein
KGPTAEPGSAT

SEQ ID NO: 35 - protein, 15 aa, Artificial Sequence
  O-glycosylation of GLP-1:Fc fusion protein
KGATAEPGSTASSGS

SEQ ID NO: 36 - protein, 15 aa, Artificial Sequence
  O-glycosylation of GLP-1:Fc fusion protein
KGPTAEAGSTASSGS

SEQ ID NO: 37 - protein, 23 aa, Artificial Sequence
  O-glycosylation of GLP-1:Fc fusion protein
KGAAPGPTPGPGSTASSGSGSAT

SEQ ID NO: 38 - protein, 23 aa, Artificial Sequence
  O-glycosylation of GLP-1:Fc fusion protein
KGAAVGATVEGGSTASSGSGSAT

SEQ ID NO: 39 - protein, 23 aa, Artificial Sequence
  O-glycosylation of GLP-1:Fc fusion protein
KGAADSTTPAPGSTASSGSGSAT

SEQ ID NO: 40 - protein, 23 aa, Artificial Sequence
  O-glycosylation of GLP-1:Fc fusion protein
KGAASLPSISSGSTASSGSGSAT

SEQ ID NO: 41 - protein, 6 aa, Artificial Sequence
  O-glycosylation sequence
PTAEPG

SEQ ID NO: 42 - protein, 11 aa, Artificial Sequence
  O-glycosylation sequence
  MISC_FEATURE (1)..(3): X is any amino acid
  MISC_FEATURE (9)..(11): X is any amino acid
XXXPAAEKXXX

SEQ ID NO: 43 - protein, 11 aa, Artificial Sequence
  O-glycosylation sequence
  MISC_FEATURE (1)..(3): X is any amino acid
  MISC_FEATURE (9)..(11): X is any amino acid
XXXPTAEPXXX